European Patent Application EP 4 353 266 A1, published April 17, 2024. Title: Ligand-binding nucleic acid complex. Applicant: Rena Therapeutics Inc. The sequence listing filed with the application follows.

SEQUENCE LISTING (12 sequences)

SEQ ID NO: 1 - DNA, 14 bp, Artificial
  Synthetic
aatgcacgtgggcc

SEQ ID NO: 2 - RNA, 14 nt, Artificial
  Synthetic
ggcccacgugcauu

SEQ ID NO: 3 - DNA, 13 bp, Artificial
  Synthetic
gcattggtattca

SEQ ID NO: 4 - RNA, 13 nt, Artificial
  Synthetic
ugaauaccaaugc

SEQ ID NO: 5 - DNA, 16 bp, Artificial
  Synthetic
acaataaataccgagg

SEQ ID NO: 6 - RNA, 16 nt, Artificial
  Synthetic
ccucgguauuuauugu

SEQ ID NO: 7 - DNA, 25 bp, Artificial
  Synthetic
ggccaaacctcggcttacctgaaat

SEQ ID NO: 8 - RNA, 26 nt, Artificial
  Synthetic
auuucagguaagccgagguuuaggcc

SEQ ID NO: 9 - RNA, 20 nt, Artificial
  Synthetic
gcacacuuccaauacuuacc

SEQ ID NO: 10 - RNA, 20 nt, Artificial
  Synthetic
gguaaguauuggaagugugc

SEQ ID NO: 11 - DNA, 16 bp, Artificial
  Synthetic
ctagttcactgaatgc

SEQ ID NO: 12 - RNA, 16 nt, Artificial
  Synthetic
gcauucagugaacuag